European Patent Specification EP 3 818 070 B1, published March 11, 2026. Title: SYNTHETIC PEPTIDES, PRODRUGS, PHARMACEUTICAL COMPOSITIONS AND USES. Applicant: Biozeus Desenvolvimento De Produtos Biofarmacêuticos do Nascimento, Caio Victor Machado França. The sequence listing filed with the application follows.

SEQUENCE LISTING (30 sequences)

SEQ ID NO: 1 - protein, 15 aa, Artificial Sequence
  Conserved region (6)...(8): Synthetic PRT based around -Ile-Ala-Trp-
RAYFWIAWYKLANSK

SEQ ID NO: 2 - protein, 15 aa, Artificial Sequence
  Conserved region (6)...(8): Synthetic PRT based around -Ile-Ala-Trp-
RQYFWIAWYKLANSA

SEQ ID NO: 3 - protein, 15 aa, Artificial Sequence
  Conserved region (6)...(8): Synthetic PRT based around -Ile-Ala-Trp-
RQAFWIAWYKLANSK

SEQ ID NO: 4 - protein, 15 aa, Artificial Sequence
  Conserved region (6)...(8): Synthetic PRT based around -Ile-Ala-Trp-
AQYFWIAWYKLANSK

SEQ ID NO: 5 - protein, 15 aa, Artificial Sequence
  Conserved region (6)...(8): Synthetic PRT based around -Ile-Ala-Trp-
RQYFWIAWYKLANSK

SEQ ID NO: 6 - protein, 15 aa, Artificial Sequence
  Conserved region (6)...(8): Synthetic PRT based around -Ile-Ala-Trp-
RQYFWIAWYKIASNK

SEQ ID NO: 7 - protein, 15 aa, Artificial Sequence
RQYFWAAWYKLANSK

SEQ ID NO: 8 - protein, 15 aa, Artificial Sequence
RQYFWIAAYKLANSK

SEQ ID NO: 9 - protein, 15 aa, Artificial Sequence
  Conserved region (6)...(8): Synthetic PRT based around -Ile-Ala-Trp-
RQYAWIAWYKLANSK

SEQ ID NO: 10 - protein, 15 aa, Artificial Sequence
  Conserved region (6)...(8): Synthetic PRT based around -Ile-Ala-Trp-
RQYFAIAWYKLANSK

SEQ ID NO: 11 - protein, 15 aa, Artificial Sequence
  Conserved region (6)...(8): Synthetic PRT based around -Ile-Ala-Trp-
RQYFWIAWAKLANSK

SEQ ID NO: 12 - protein, 15 aa, Artificial Sequence
  Conserved region (6)...(8): Synthetic PRT based around -Ile-Ala-Trp-
RQYFWIAWYALANSK

SEQ ID NO: 13 - protein, 15 aa, Artificial Sequence
  Conserved region (6)...(8): Synthetic PRT based around -Ile-Ala-Trp-
RQYFWIAWYKLAASK

SEQ ID NO: 14 - protein, 15 aa, Artificial Sequence
  Conserved region (6)...(8): Synthetic PRT based around -Ile-Ala-Trp-
RQYFWIAWYKLANAK

SEQ ID NO: 15 - protein, 15 aa, Artificial Sequence
  Conserved region (6)...(8): Synthetic PRT based around -Ile-Ala-Trp-
EQYFWIAWYKIANSK

SEQ ID NO: 16 - protein, 15 aa, Artificial Sequence
  Conserved region (6)...(8): Synthetic PRT based around -Ile-Ala-Trp-
RQYFWIAWYKIANSE

SEQ ID NO: 17 - protein, 13 aa, Artificial Sequence
  Conserved region (5)...(7): Synthetic PRT based around -Ile-Ala-Trp-
QYFWIAWYKLANS

SEQ ID NO: 18 - protein, 11 aa, Artificial Sequence
  Conserved region (4)...(6): Synthetic PRT based around -Ile-Ala-Trp-
YFWIAWYKLAN

SEQ ID NO: 19 - protein, 9 aa, Artificial Sequence
  Conserved region (3)...(5): Synthetic PRT based around -Ile-Ala-Trp-
FWIAWYKLA

SEQ ID NO: 20 - protein, 9 aa, Artificial Sequence
  Conserved region (6)...(8): Synthetic PRT based around -Ile-Ala-Trp-
RQYFWIAWY

SEQ ID NO: 21 - protein, 9 aa, Artificial Sequence
  Conserved region (3)...(5): Synthetic PRT based around -Ile-Ala-Trp-
YWIAWYKLL

SEQ ID NO: 22 - protein, 8 aa, Artificial Sequence
  Conserved region (6)...(8): Synthetic PRT based around -Ile-Ala-Trp-
RQYFWIAW

SEQ ID NO: 23 - protein, 7 aa, Artificial Sequence
  Conserved region (2)...(4): Synthetic PRT based around -Ile-Ala-Trp-
WIAWYKL

SEQ ID NO: 24 - protein, 5 aa, Artificial Sequence
  Conserved region (1)...(3): Synthetic PRT based around -Ile-Ala-Trp-
IAWYK

SEQ ID NO: 25 - protein, 5 aa, Artificial Sequence
  Conserved region (1)...(3): Synthetic PRT based around -Ile-Ala-Trp-
IAWYE

SEQ ID NO: 26 - protein, 5 aa, Artificial Sequence
IAYYK

SEQ ID NO: 27 - protein, 18 aa, Artificial Sequence
  Conserved region (9)...(11): Synthetic PRT based around -Ile-Ala-Trp-
GERRQYFWIAWYKLANSK

SEQ ID NO: 28 - protein, 15 aa, Artificial Sequence
  Conserved region (1)...(3) AND (11)...(13): synthetic PRT based around -Ile-Ala-Trp-
  misc_feature (6)...(10): amino acid is optionally linked to poly-Gly linkers
IAWYKGGGGGIAWYK

SEQ ID NO: 29 - protein, 17 aa, Artificial Sequence
  Conserved region (1)...(3): synthetic PRT based around -Ile-Ala-Trp-
  misc_feature (7)...(11): amino acid is optionally linked to poly-Gly linkers
IAWYKRGGGGGRKYWAI

SEQ ID NO: 30 - protein, 25 aa, Artificial Sequence
  Conserved region (1)...(3) AND (11)...(13) AND (21)...(23): synthetic PRT based around -Ile-Ala-Trp-
  misc_feature (6)...(10) AND (16)...(20): amino acid is optionally linked to poly-Gly linkers
IAWYKGGGGGIAWYKGGGGGIAWYK